European Patent Specification EP 4 056 689 B1, published November 1, 2023. Title: Novel asparagine synthase variant and a method for producing L-valine using the same. Applicant: CJ CheilJedang Corporation. The sequence listing filed with the application follows.

SEQUENCE LISTING (11 sequences)

SEQ ID NO: 1 - protein, 613 aa, Artificial Sequence
  Asparagine synthase variant
MRHRGPDDAGTWHDADAAFGFNRLSIIDIAHSHQPLRWGPTDEPDRYAMTFNGEIYNYVELRKELSDLGYTFNTSGDGEPIVVGFHHWGESVVEHLRGMFGIAIWDTKEKSLFLARDQFGIKPLFYATTEHGTVFSSEKKTILEMAEEMNLDLGLDKRTIEHYVDLQYVPEPDTLHAQISRLESGCTATVRLGGKLEQKRYFKPQFPVQKVVKGKEQDLFDRIAQVLEDSVEKHMRADVTVGSFLSGGIDSTAIAALAKRHNPDLLTFTTGFEREGYSEVDVAAESAAAIGTEHIVKIVSPEEYANAIPKIMWYLDDPVADPSLVPLYFVAAEARKHVKVVLSGEGADELFGGYTIYKEPLSLAPFEKIPSPLRKGLGKLSKVLPDGMKGKSLLERGSMTMEERYYGNARSFNFEQMQRVIPWAKREWDHREVTAPIYAQSRNFDPVARMQHLDLFTWMRGDILVKADKINMANSLELRVPFLDKEVFKVAETIPYDLKIANGTTKYALRRALEQIVPPHVLHRKKLGFPVPMRHWLAGDELFGWAQDAIKESGTEDIFNKQAVLDMLNEHRDGVSDHSRRLWTVLSFMVWHGIFVENRIDPQIEDRSYPVEL

SEQ ID NO: 2 - DNA, 1842 bp, Artificial Sequence
  Asparagine synthase variant coding gene
atgcgccaccgtggtcctgacgatgccggcacttggcatgacgccgatgcagcgtttggattcaaccgcctctccatcattgatattgcacactcccaccaaccactgcgttggggacctacggatgaacccgaccgctacgcaatgactttcaacggtgagatctacaactacgttgagctgcgtaaagagctctcggatttgggatatacctttaatacttctggcgatggcgagccaattgttgtcggtttccaccactggggcgagtccgtggtcgagcatctccgcggaatgttcggcattgccatttgggatacaaaggaaaagtcgcttttccttgcgcgtgatcagttcggcatcaagccactgttctacgcaaccaccgagcatggcaccgtgttctcctcagagaagaagaccatcttggagatggccgaggagatgaatctagatctgggccttgataagcgcaccattgagcactacgtggacttgcagtacgtgcccgagccagatacccttcacgcgcagatttcccgcttggagtcaggctgcaccgcaacagttcgtctgggcggcaagctggaacagaagcgttacttcaagcctcagttcccagtacagaaggtcgtaaagggtaaggagcaggacctcttcgatcgcattgcccaggtgttggaggatagcgtcgaaaagcatatgcgtgccgacgtgaccgtaggctcgttcctttccggcggcattgattcaaccgcaattgcggcgcttgcaaagcgccacaaccctgacctgctcaccttcaccaccggtttcgagcgtgaaggctactcggaggtcgatgtggctgcggagtccgccgctgcgattggcactgagcacatcgtgaagattgtctcgcctgaggaatacgccaacgcgattcctaagatcatgtggtacttggatgatcctgtagctgacccatcattggtcccgctgtacttcgtggcagcggaagcacgtaagcacgtcaaggttgtgctgtctggcgagggcgcagatgagctgttcggtggatacaccatttacaaggagccgctatcgcttgctccatttgagaagatcccttccccactacgtaaaggcctgggaaagctcagcaaggttctgccagacggcatgaagggcaagtcccttcttgagcgtggctccatgaccatggaagagcgctactacggcaacgctcgctccttcaatttcgagcagatgcaacgcgttattccatgggcaaagcgcgaatgggaccaccgcgaagtcactgcgccgatctacgcacagtcccgcaactttgatccagtagcccgcatgcaacacctggatctgttcacctggatgcgcggcgacatcctggtcaaggctgacaagatcaacatggcgaactcccttgagctgcgagttccattcttggataaagaagttttcaaggttgcagagaccattccttacgatctgaagattgccaacggtaccaccaagtacgcgctgcgcagggcactcgagcagattgttccgcctcacgttttgcaccgcaagaagctgggcttccctgttcccatgcgccactggcttgccggcgatgagctgttcggttgggcgcaggacgccatcaaggaatccggtactgaagatatcttcaacaagcaggctgtgctggatatgctgaacgagcaccgcgatggcgtgtcagatcattcccgtcgactgtggactgttctgtcatttatggtgtggcacggcatttttgtggaaaaccgcattgatccacagattgaggaccgctcctacccagtcgagctttaa

SEQ ID NO: 3 - protein, 613 aa, Artificial Sequence
  Wild-type asparagine synthase
MRHRGPDDAGTWHDADAAFGFNRLSIIDIAHSHQPLRWGPTDEPDRYAMTFNGEIYNYVELRKELSDLGYTFNTSGDGEPIVVGFHHWGESVVEHLRGMFGIAIWDTKEKSLFLARDQFGIKPLFYATTEHGTVFSSEKKTILEMAEEMNLDLGLDKRTIEHYVDLQYVPEPDTLHAQISRLESGCTATVRPGGKLEQKRYFKPQFPVQKVVKGKEQDLFDRIAQVLEDSVEKHMRADVTVGSFLSGGIDSTAIAALAKRHNPDLLTFTTGFEREGYSEVDVAAESAAAIGTEHIVKIVSPEEYANAIPKIMWYLDDPVADPSLVPLYFVAAEARKHVKVVLSGEGADELFGGYTIYKEPLSLAPFEKIPSPLRKGLGKLSKVLPDGMKGKSLLERGSMTMEERYYGNARSFNFEQMQRVIPWAKREWDHREVTAPIYAQSRNFDPVARMQHLDLFTWMRGDILVKADKINMANSLELRVPFLDKEVFKVAETIPYDLKIANGTTKYALRRALEQIVPPHVLHRKKLGFPVPMRHWLAGDELFGWAQDAIKESGTEDIFNKQAVLDMLNEHRDGVSDHSRRLWTVLSFMVWHGIFVENRIDPQIEDRSYPVEL

SEQ ID NO: 4 - DNA, 1842 bp, Artificial Sequence
  Wild-type asparagine synthase coding gene
atgcgccaccgtggtcctgacgatgccggcacttggcatgacgccgatgcagcgtttggattcaaccgcctctccatcattgatattgcacactcccaccaaccactgcgttggggacctacggatgaacccgaccgctacgcaatgactttcaacggtgagatctacaactacgttgagctgcgtaaagagctctcggatttgggatatacctttaatacttctggcgatggcgagccaattgttgtcggtttccaccactggggcgagtccgtggtcgagcatctccgcggaatgttcggcattgccatttgggatacaaaggaaaagtcgcttttccttgcgcgtgatcagttcggcatcaagccactgttctacgcaaccaccgagcatggcaccgtgttctcctcagagaagaagaccatcttggagatggccgaggagatgaatctagatctgggccttgataagcgcaccattgagcactacgtggacttgcagtacgtgcccgagccagatacccttcacgcgcagatttcccgcttggagtcaggctgcaccgcaacagttcgtccgggcggcaagctggaacagaagcgttacttcaagcctcagttcccagtacagaaggtcgtaaagggtaaggagcaggacctcttcgatcgcattgcccaggtgttggaggatagcgtcgaaaagcatatgcgtgccgacgtgaccgtaggctcgttcctttccggcggcattgattcaaccgcaattgcggcgcttgcaaagcgccacaaccctgacctgctcaccttcaccaccggtttcgagcgtgaaggctactcggaggtcgatgtggctgcggagtccgccgctgcgattggcactgagcacatcgtgaagattgtctcgcctgaggaatacgccaacgcgattcctaagatcatgtggtacttggatgatcctgtagctgacccatcattggtcccgctgtacttcgtggcagcggaagcacgtaagcacgtcaaggttgtgctgtctggcgagggcgcagatgagctgttcggtggatacaccatttacaaggagccgctatcgcttgctccatttgagaagatcccttccccactacgtaaaggcctgggaaagctcagcaaggttctgccagacggcatgaagggcaagtcccttcttgagcgtggctccatgaccatggaagagcgctactacggcaacgctcgctccttcaatttcgagcagatgcaacgcgttattccatgggcaaagcgcgaatgggaccaccgcgaagtcactgcgccgatctacgcacagtcccgcaactttgatccagtagcccgcatgcaacacctggatctgttcacctggatgcgcggcgacatcctggtcaaggctgacaagatcaacatggcgaactcccttgagctgcgagttccattcttggataaagaagttttcaaggttgcagagaccattccttacgatctgaagattgccaacggtaccaccaagtacgcgctgcgcagggcactcgagcagattgttccgcctcacgttttgcaccgcaagaagctgggcttccctgttcccatgcgccactggcttgccggcgatgagctgttcggttgggcgcaggacgccatcaaggaatccggtactgaagatatcttcaacaagcaggctgtgctggatatgctgaacgagcaccgcgatggcgtgtcagatcattcccgtcgactgtggactgttctgtcatttatggtgtggcacggcatttttgtggaaaaccgcattgatccacagattgaggaccgctcctacccagtcgagctttaa

SEQ ID NO: 5 - DNA, 36 bp, Artificial Sequence
  ltsA_1F
tcgagctcggtacccctccatcattgatattgcaca

SEQ ID NO: 6 - DNA, 44 bp, Artificial Sequence
  ltsA_2R
ttctgttccagcttgccgcccagacgaactgttgcggtgcagcc

SEQ ID NO: 7 - DNA, 44 bp, Artificial Sequence
  ltsA_3F
ggctgcaccgcaacagttcgtctgggcggcaagctggaacagaa

SEQ ID NO: 8 - DNA, 36 bp, Artificial Sequence
  ltsA_4R
ctctagaggatcccccttgacgtgcttacgtgcttc

SEQ ID NO: 9 - DNA, 21 bp, Artificial Sequence
  ltsA_5F
ctccatcattgatattgcaca

SEQ ID NO: 10 - DNA, 21 bp, Artificial Sequence
  ltsA_6R
cttgacgtgcttacgtgcttc

SEQ ID NO: 11 - DNA, 5803 bp, Artificial Sequence
  pDCM2
gttcgcttgctgtccataaaaccgcccagtctagctatcgccatgtaagcccactgcaagctacctgctttctctttgcgcttgcgttttcccttgtccagatagcccagtagctgacattcatccggggtcagcaccgtttctgcggactggctttctacgtgttccgcttcctttagcagcccttgcgccctgagtgcttgcggcagcgtgaagctagcttttatcgccattcgccattcaggctgcgcaactgttgggaagggcgatcggtgcgggcctcttcgctattacgccagctggcgaaagggggatgtgctgcaaggcgattaagttgggtaacgccagggttttcccagtcacgacgttgtaaaacgacggccagtgaattcgagctcggtacccggggatcctctagagtcgacctgcaggcatgcaagcttggcgtaatcatggtcatagctgtttcctgtgtgaaattgttatccgctcacaattccacacaacatacgagccggaagcataaagtgtaaagcctggggtgcctaatgagtgagctaactcacattaattgcgttgcgctcactgcccgctttccagtcgggaaacctgtcgtgccagctgcattaatgaatcggccaacgcgcggggagaggcggtttgcgtattgggcgctcttccgcttcctcgctcactgactcgctgcgctcggtcgttcggctgcggcgagcggtatcagctcactcaaaggcggtaatacggttatccacagaatcaggggataacgcaggaaagaacatgtgagcaaaaggccagcaaaaggccaggaaccgtaaaaaggccgcgttgctggcgtttttccataggctccgcccccctgacgagcatcacaaaaatcgacgctcaagtcagaggtggcgaaacccgacaggactataaagataccaggcgtttccccctggaagctccctcgtgcgctctcctgttccgaccctgccgcttaccggatacctgtccgcctttctcccttcgggaagcgtggcgctttctcaatgctcacgctgtaggtatctcagttcggtgtaggtcgttcgctccaagctgggctgtgtgcacgaaccccccgttcagcccgaccgctgcgccttatccggtaactatcgtcttgagtccaacccggtaagacacgacttatcgccactggcagcagccactggtaacaggattagcagagcgaggtatgtaggcggtgctacagagttcttgaagtggtggcctaactacggctacactagaaggacagtatttggtatctgcgctctgctgaagccagttaccttcggaaaaagagttggtagctcttgatccggcaaacaaaccaccgctggtagcggtggtttttttgtttgcaagcagcagattacgcgcagaaaaaaaggatctcaagaagatcctttgatcttttctacggggtctgacgctcagtggaacgaaaactcacgttaagggattttggtcatgagattatcaaaaaggatcttcacctagatccttttggggtgggcgaagaactccagcatgagatccccgcgctggaggatcatccagccctgatagaaacagaagccactggagcacctcaaaaacaccatcatacactaaatcagtaagttggcagcatcacccgacgcactttgcgccgaataaatacctgtgacggaagatcacttcgcagaataaataaatcctggtgtccctgttgataccgggaagccctgggccaacttttggcgaaaatgagacgttgatcggcacgtaagaggttccaactttcaccataatgaaataagatcactaccgggcgtattttttgagttatcgagattttcaggagctgatagaaacagaagccactggagcacctcaaaaacaccatcatacactaaatcagtaagttggcagcatcacccgacgcactttgcgccgaataaatacctgtgacggaagatcacttcgcagaataaataaatcctggtgtccctgttgataccgggaagccctgggccaacttttggcgaaaatgagacgttgatcggcacgtaagaggttccaactttcaccataatgaaataagatcactaccgggcgtattttttgagttatcgagattttcaggagctctttggcatcgtctctcgcctgtcccctcagttcagtaatttcctgcatttgcctgtttccagtcggtagatattccacaaaacagcagggaagcagcgcttttccgctgcataaccctgcttcggggtcattatagcgattttttcggtatatccatcctttttcgcacgatatacaggattttgccaaagggttcgtgtagactttccttggtgtatccaacggcgtcagccgggcaggataggtgaagtaggcccacccgcgagcgggtgttccttcttcactgtcccttattcgcacctggcggtgctcaacgggaatcctgctctgcgaggctggccggctaccgccggcgtaacagatgagggcaagcggatggctgatgaaaccaagccaaccaggaagggcagcccacctatcaaggtgtactgccttccagacgaacgaagagcgattgaggaaaaggcggcggcggccggcatgagcctgtcggcctacctgctggccgtcggccagggctacaaaatcacgggcgtcgtggactatgagcacgtccgcgagggcgtcccggaaaacgattccgaagcccaacctttcatagaaggcggcggtggaatcgaaatctcgtgatggcaggttgggcgtcgcttggtcggtcatttcgaaaaaggttaggaatacggttagccatttgcctgcttttatatagttcantatgggattcacctttatgttgataagaaataaaagaaaatgccaataggatatcggcattttcttttgcgtttttatttgttaactgttaattgtccttgttcaaggatgctgtctttgacaacagatgttttcttgcctttgatgttcagcaggaagctcggcgcaaacgttgattgtttgtctgcgtagaatcctctgtttgtcatatagcttgtaatcacgacattgtttcctttcgcttgaggtacagcgaagtgtgagtaagtaaaggttacatcgttaggcggatcaagatccatttttaacacaaggccagttttgttcagcggcttgtatgggccagttaaagaattagaaacataaccaagcatgtaaatatcgttagacgtaatgccgtcaatcgtcatttttgatccgcgggagtcagtgaacaggtaccatttgccgttcattttaaagacgttcgcgcgttcaatttcatctgttactgtgttagatgcaatcagcggtttcatcacttttttcagtgtgtaatcatcgtttagctcaatcataccgagagcgccgtttgctaactcagccgtgcgttttttatcgctttgcagaagtttttgactttcttgacggaagaatgatgtgcttttgccatagtatgctttgttaaataaagattcttcgccttggtagccatcttcagttccagtgtttgcttcaaatactaagtatttgtggcctttatcttctacgtagtgaggatctctcagcgtatggttgtcgcctgagctgtagttgccttcatcgatgaactgctgtacattttgatacgtttttccgtcaccgtcaaagattgatttataatcctctacaccgttgatgttcaaagagctgtctgatgctgatacgttaacttgtgcagttgtcagtgtttgtttgccgtaatgtttaccggagaaatcagtgtagaataaacggatttttccgtcagatgtaaatgtggctgaacctgaccattcttgtgtttggtcttttaggatagaatcatttgcatcgaatttgtcgctgtctttaaagacgcggccagcgtttttccagctgtcaatagaagtttcgccgactttttgatagaacatgtaaatcgatgtgtcatccgcatttttaggatctccggctaatgcaaagacgatgtggtagccgtgatagtttgcgacagtgccgtcagcgttttgtaatggccagctgtcccaaacgtccaggccttttgcagaagagatatttttaattgtggacgaatcaaattcagaaacttgatatttttcatttttttgctgttcagggatttgcagcatatcatggcgtgtaatatgggaaatgccgtatgtttccttatatggcttttggttcgtttctttcgcaaacgcttgagttgcgcctcctgccagcagtgcggtagtaaaggttaatactgttgcttgttttgcaaactttttgatgttcatcgttcatgtctccttttttatgtactgtgttagcggtctgcttcttccagccctcctgtttgaagatggcaagttagttacgcacaataaaaaaagacctaaaatatgtaaggggtgacgccaaagtatacactttgccctttacacattttaggtcttgcctgctttatcagtaacaaacccgcgcgatttacttttcgacctcattctattagactctcgtttggattgcaactggtctattttcctcttttgtttgatagaaaatcataaaaggatttgcagactacgggcctaaagaactaaaaaatctatctgtttcttttcattctctgtattttttatagtttctgttgcatgggcataaagttgcctttttaatcacaattcagaaaatatcataatatctcatttcactaaataatagtgaacggcaggtatatgtgatgggttaaaaaggatcaccccagagtcccgctcagaagaactcgtcaagaaggcgatagaaggcgatgcgctgcgaatcgggagcggcgataccgtaaagcacgaggaagcggtcagcccattcgccgccaagctcttcagcaatatcacgggtagccaacgctatgtcctgatagcggtccgccacacccagccggccacagtcgatgaatccagaaaagcggccattttccaccatgatattcggcaagcaggcatcgccatgggtcacgacgagatcctcgccgtcgggcatccgcgccttgagcctggcgaacagttcggctggcgcgagcccctgatgctcttcgtccagatcatcctgatcgacaagaccggcttccatccgagtacgtgctcgctcgatgcgatgtttcgcttggtggtcgaatgggcaggtagccggatcaagcgtatgcagccgccgcattgcatcagccatgatggatactttctcggcaggagcaaggtgagatgacaggagatcctgccccggcacttcgcccaatagcagccagtcccttcccgcttcagtgacaacgtcgagacagctgcgcaaggaacgcccgtcgtggccagccacgatagccgcgctgcctcgtcttggagttcattcagggcaccggacaggtcggtcttgacaaaaagaaccgggcgcccctgcgctgacagccggaacacggcggcatcagagcagccgattgtctgttgtgcccagtcatagccgaatagcctctccacccaagcggccggagaacctgcgtgcaatccatcttgttcaatcatgcgaaacgatcctcatcctgtctcttgatcagatcttgatcccctgcgccatcagatccttggcggcaagaaagccatccagtttactttgcagggcttcccaaccttaccagagggcgccccagctggcaattccg